European Patent Application EP 4 481 050 A1, published December 25, 2024. Title: GENE-MODIFIED MICROORGANISM FOR PRODUCING 3-HYDROXYADIPIC ACID, ALPHA-HYDROMUCONIC ACID, AND/OR ADIPIC ACID, AND PRODUCTION METHOD FOR SAID CHEMICAL PRODUCTS. Applicant: 東レ株式会社. Application JP. The sequence listing filed with the application follows.

SEQUENCE LISTING (47 sequences)

SEQ ID NO: 1 - protein, 312 aa, Serratia grimesii NBRC13537
MKVAVLGAAGGIGQALALLLKTQLPSGSELSLYDIAPVTPGVAVDLSHIPTAVKIKGFSGEDATPALHGADVVLISAGVARKPGMDRSDLFNVNAGIVRNLIQQVATTCPKACIGIITNPVNTTVAIAAEVLKKAGVYDKNKLFGVTSLDIIRSNTFVAELKGKQPEELNVPVIGGHSGVTILPLLSQIPGVSFTEQEVADLTKRIQNAGTEVVEAKAGGGSATLSMGQAAARFGLSLVRALQGEKGVVECAYVEGDGKYARFFAQPLVLGKNGVEERKDIGTLSAFEQKALTDMLDVLHKDIELGEKFINN

SEQ ID NO: 2 - protein, 915 aa, Serratia grimesii NBRC13537
MGLSSCVLPQNTGRQAPKQTIRQIRNTTMSERLNNDVDPIETRDWLQAIESVIREEGVERAQFLIDQVLGEARKGGVSVAAGAAAHNYVNTIAVEDEPAYPGNLDLERRIRSAIRWNAVMTVLRASKKDLDLGGHMASFQSSATFYEVCFNHFFRARNEQDGGDLVYFQGHISPGVYARAFLEGRLTEDQMNNFRQEVHGKGLSSYPHPKLMPEFWQFPTVSMGLGPISAIYQAKFLKYLEHRGLKNTSAQTVYAFLGDGEMDEPESKGAITIATREKLDNLVFVINCNLQRLDGPVTGNGKIINELEGIFAGAGWQVLKVIWGGRWDELLRKDTSGKLIQLMNETLDGDYQTFKSKDGAYVREHFFGRFPETAALVKDMTDDEIWALNRGGHDPKKVFAALKKAQDTQGKPTVILAHTIKGYGMGETAEGKNIAHQVKKMNMEGVHHFRDRFNVPVADADIEKLPYITFEKESEEYKYLHERRQALKGYVPTRLPAFTQKLEMPALEDFSSLLEEQNKEISTTIAFVRALNVMLKNKSIKDRLVPIIADEARTFGMEGLFRQIGIYSPNGQQYTPQDREQVAYYKEDEKGQILQEGINELGAASSWLAAATSYSTNDLPMIPFYIYYSMFGFQRIGDLCWAAGDQQARGFLIGGTSGRTTLNGEGLQHEDGHSHIQSLTIPNCISYDPAYAYEVAVIMHDGLVRMYGDAQENVYYYITTLNENYHMPAMPQGAEEGIRKGIYKLDTLAGSKGKVQLLGSGSILRHVRDAAKILADDYGVGSDIYSVTSFTELARDGQDCERWNMLHPTETPRVPYIAQVMNDAPAVASTDYMKLFAEQVRTYVPASDYRVLGTDGFGRSDSRENLRHHFEVDASYVVVAALGELAKRGEIEASVVADAIKKFDINPEKVNPRLA

SEQ ID NO: 3 - protein, 626 aa, Serratia grimesii NBRC13537
MSIEIKVPDIGADEVEITEILVKVGDKVEAEQSLITVEGDKASMEVPSPQAGVVKEIKVSVGDKTETGKLLMIFEAEGAAAAAPAAKAEEKPAAAPAAPAAAAAKDVAVPDIGADEVEVTEILVKVGDKVEAEQSLITVEGDKASMEVPAPFAGTVKEIKIGTGDKVTTGSLIMVFEVAGAASAAAPAAAQAPAAPAAPAASAAKDVAVPDIGGDEVEVTEVMVKVGDKVAAEQSLITVEGDKASMEVPAPFAGTVKEIKISAGDKVKTGSLIMVFEVEGAAPAAAPAQKAEAAPAPAASSAPAPQAAPAAKGEFAENDAYVHATPVIRRLAREFGVNLAKVKGTGRKGRILREDVQTYVKDAVKRAEAAPTAAAGGGLPGMLPWPKVDFSKFGEIEEVELGRIQKISGANLSRNWVMIPHVTHFDKTDITDLEAFRKQQNEEAAKRKLDVKFTPVVFIMKAVAAALEQMPRFNSSLSEDGQKLTLKKYINVGVAVDTPNGLVVPVFKDVNKKSITELSRELMAISKKARDGKLTAGEMQGGCFTISSLGGIGTTHFAPIVNAPEVAILGVSKSAMEPVWNGKEFVPRLMMPMSLSFDHRVIDGADGARFITIINNMLADIRRMVM

SEQ ID NO: 4 - protein, 475 aa, Serratia grimesii NBRC13537
MMSTEIKTQVVVLGAGPAGYSAAFRCADLGLETVLVERYSTLGGVCLNVGCIPSKALLHVAKVIEEAKALAEHGIVFGEPKTDIDKVRVWKEKVINQLTGGLAGMAKGRKVKVVNGLGKFTGANTLVVEGENGPTTINFDNAIIAAGSRPIQLPFIPHEDPRVWDSTDALELKTVPERLLVMGGGIIGLEMGTVYHALGSQIDVVEMFDQVIPAADKDVVKVFTKRISKQFNLMLETKVTAVEAKEDGIYVTMEGKKAPAEPQRYDAVLVAIGRVPNGKLLEAGKAGVEVDERGFINVDKQLRTNVPHIFAIGDIVGQPMLAHKGVHEGHVAAEVIAGMKHYFDPKVIPSIAYTEPEVAWVGLTEKEAKEKGISYETSTFPWAASGRAIASDCADGMTKLIFDKETHRIIGGAIVGTNGGELLGEIGLAIEMGCDAEDIALTIHAHPTLHESVGLAAEIYEGSITDLPNPKAKKK

SEQ ID NO: 5 - protein, 272 aa, Serratia grimesii NBRC13537
LKLVLPIDSAPFAEKNSPMAYSKIRQPKLSDVIEQQLEHLILEGTLRPGEKLPPERELAKQFDVSRPSLREAIQRLEAKGLLLRRQGGGTFVQTNLWQSFSDPLAELLADHPESQFDLLETRHALEGIAAYYAALRGTDEDLARIRDCHIVIQQAQDSGDLDAEADAVMQYQIAVTEAAHNVVLLHLLRCMGPMLEQNVRQNFELLYSRREMLAKVSSHRAGIFEAIVAREPEKAREASHRHLAFIEEILLDLSREHTRRERSLRRLQQRKD

SEQ ID NO: 6 - protein, 760 aa, Serratia grimesii NBRC13537
MTELNEKLAKAWEGFSKGDWQKEVNVRDFIQKNYTPYEGDESFLAGATEATSTLWEKVMEGIKLENRTHAPVDFDTNVAATITSHDAGYIAKELETIVGLQTDAPLKRALIPFGGIKMVEGSCKVYGRELDPQLKKVFTEYRKTHNQGVFDVYTKDILNCRKSGVLTGLPDAYGRGRIIGDYRRVALYGIDFLMADKLNQFKSLQTKLENGEDLEMTIQLREEIAEQHRALGQIKEMAAKYGYDISGPATTAQEAVQWTYFGYLAAVKSQNGAAMSFGRVSTFLDVFIQRDIEAGKLNEEQAQELIDHLVMKLRMVRFLRTPEYDELFSGDPIWATESLAGMGVDGRTLVTKNSFRFLNTLYTMGPSPEPNMTILWSEKLPLNFKKYAAKVSIDTSSVQYENDDLMRPDFNNDDYAIACCVSPMIVGKQMQFFGARANLAKTMLYAINGGVDEKLKIQVGPKEAPMMDTVLDYDKVMERMDHFMDWLAKQYVTALNIIHYMHDKYSYEAALMALHDRDVYRTMACGIAGLSVAADSLSAIKYAKVSTIRDEDGLAVDFKIEGEYPQFGNNDARVDDIACDLVERFMKKIQKLRTYRNAVATQSVLTITSNVVYGKKTGNTPDGRRAGAPFGPGANPMHGRDQKGAVASLTSVAKLPFAYAKDGISYTFSIVPNALGKDDDVRKANLAGLMDGYFHHEASIEGGQHLNVNVMNREMLLDAMENPEKYPQLTIRVSGYAVRFNSLTKEQQQDVITRTFTQSM

SEQ ID NO: 7 - protein, 256 aa, Serratia grimesii NBRC13537
LTVNIGENPAMSVKGRIHSFESCGTVDGPGIRFIVFFQGCLMRCLYCHNRDTWDTHGGKEVTVEELMKDTVSYRHFMNASGGGVTASGGEAILQAEFVRDWFRACHAEGISTCLDTNGFVRRYDPVIDELLDATDLVMLDLKQMNDDIHQNLVGVSNHRTLDFARYLAKRNQRTWIRYVVVPGWSDDDASTHLLGEFTKGMTNIEKIELLPYHELGKHKWVAMGEEYKLDGVHPPKADTMERVKGILESYGHKVMY

SEQ ID NO: 8 - DNA, 200 bp, Escherichia coli str. K-12 substr. MG1655
  source 1..200: mol_type = genomic DNA
cgtaattgccctttaaaattcggggcgccgaccccatgtggtctcaagcccaaaggaagagtgaggcgagtcagtcgcgtaatgcttaggcacaggattgatttgtcgcaatgattgacacgattccgcttgacgctgcgtaaggtttttgtaattttacaggcaaccttttattcactaacaaatagctggtggaatat

SEQ ID NO: 9 - DNA, 30 bp, synthetic construct
  source 1..30: mol_type = other DNA
taccgtcgacctcgacgtaattgcccttta

SEQ ID NO: 10 - DNA, 41 bp, synthetic construct
  source 1..41: mol_type = other DNA
ggccccccctcgagtcattaagtactatattccaccagcta

SEQ ID NO: 11 - DNA, 32 bp, synthetic construct
  source 1..32: mol_type = other DNA
ctggtggaatatatgcacgacgtattcatctg

SEQ ID NO: 12 - DNA, 41 bp, synthetic construct
  source 1..41: mol_type = other DNA
ctcgagtcattaagtgttaactcaaacccgctcgatggcca

SEQ ID NO: 13 - DNA, 55 bp, synthetic construct
  source 1..55: mol_type = other DNA
gagcgggtttgagttcaattgtagctggtggaatatttgatcaataaaacgtacg

SEQ ID NO: 14 - DNA, 34 bp, synthetic construct
  source 1..34: mol_type = other DNA
gagtcattaagtgtttcacttgatcagcggcacg

SEQ ID NO: 15 - DNA, 1530 bp, synthetic construct
  source 1..1530: mol_type = other DNA
atggcagaaagtaatgcggcaattcaatcggctgcgattatcggcgcgggaacgatgggcagaggcatcgcttatcttttcgcgcaaaaaggcattcgcacggtgctttataatcgcaacggcaataccctcaatcaggctcgcgaatatatcgcgcaagacctgaacaagaaagtcgaacagggcaagatcgcgctgcaggataaaggcgcggtgctggccaatctaatgttcacttcagtgtttgaggccatcgccgacagcgagctggtgatagaaaccatcgccgagcaagaacaaaccaaacttgaggtgctggcggccatcgccgcggtggtcaagcccgacacgctgatcgccaccaatacctcctcactgtcgcttaacaagctggctactgcggtgacgcacagcgaacgctttatcggtttgcattttttcaaccccgcgccgctgatgaagctgattgaaatcattccggcctactttaccgcgcacgccaccaccgaacgctgccgccaactggtggcggcgttggggaaacacgatgtcgtctgccaggccacgccggggttcatcgtcaatcgcatggcccgcccctactacctggaagggttccgcctgttggaagaacacgtggcgcgcgcggctcagatcgaccgcgccctcaaggccggcgggcgcttccgcatggggccgctcgagctgaccgattttatcggccaagacatcaactatcaggtcagtcggcaaatctggcaggatatgcaatacgacccgcgctatacccccggtcatctgcagcgttcactggtcgatgccggtctgttggggaaaaagaacggccgctcctattttgccgccgaagaaaccgccccgccggtgacggccgccagcaatgcagacgtcgagacgctgcgcgtttacggcgagcaccctttttttaccctgttacagcagcgagccgcgcttcagtggccacagctgcgcgtggaacaacggccggcattaccggggctggggtcggccgtccagatcaatgacgctttcaccgtcagcatcaccgatggccgcacggcgagccaactggccgagcagacggcagcggatgcctttgtggtcgatgtcgccctgaactacgccgacacgacgtatctggcggcggcgcacagccgccacgcctctgcggccaataaggcgctgtttttacgcctgctgcacacggcaatcccgcaggttgaatttatcaaggactctccggcgcttatcgtcgcccgcgtcctcagcagcctgatcaatgagtcggtgatcatggtggaaagcggcgtctgcagccgggaagacatcgatgtcgccgccgtcgcgggcgttaactacgccggcggcattttcgactggctcggcaaactgggggagaaaaacgtcaggacaacgctgagcaatctggctcagctgctgcacgcggcgcgctatgcgccgcattacacccttctgcacgccgcgcaaccggcgctgacgaccacgccttaa

SEQ ID NO: 16 - DNA, 35 bp, synthetic construct
  source 1..35: mol_type = other DNA
ctggtggaatatagtactatggcagaaagtaatgc

SEQ ID NO: 17 - DNA, 39 bp, synthetic construct
  source 1..39: mol_type = other DNA
ttccaccagctaagtgctagcttaaggcgtggtcgtcag

SEQ ID NO: 18 - DNA, 40 bp, synthetic construct
  source 1..40: mol_type = other DNA
cggccagtgaattcgagctccgtaattgccctttaaaatt

SEQ ID NO: 19 - DNA, 41 bp, synthetic construct
  source 1..41: mol_type = other DNA
gatccccgggtaccgcatgctatattccaccagctatttgt

SEQ ID NO: 20 - DNA, 34 bp, synthetic construct
  source 1..34: mol_type = other DNA
ggtggaatatggatcatgaaagtcgcagtcctcg

SEQ ID NO: 21 - DNA, 34 bp, synthetic construct
  source 1..34: mol_type = other DNA
ctcccaattgggatccttacttattaacgaactc

SEQ ID NO: 22 - DNA, 70 bp, synthetic construct
  source 1..70: mol_type = other DNA
gaaattggtaagaccaattgacttcggcaagtggcttaagacaggaactcgtgtaggctggagctgcttc

SEQ ID NO: 23 - DNA, 70 bp, synthetic construct
  source 1..70: mol_type = other DNA
tatgcgcttgatttacaacatcttctggataatttttaccagaaaaatcaatgggaattagccatggtcc

SEQ ID NO: 24 - DNA, 20 bp, synthetic construct
  source 1..20: mol_type = other DNA
cggtgccctgaatgaactgc

SEQ ID NO: 25 - DNA, 18 bp, synthetic construct
  source 1..18: mol_type = other DNA
agtgatgcgtgtgtaagt

SEQ ID NO: 26 - DNA, 18 bp, synthetic construct
  source 1..18: mol_type = other DNA
aaatggttgcggaagact

SEQ ID NO: 27 - DNA, 40 bp, synthetic construct
  source 1..40: mol_type = other DNA
cggccagtgaattcgagctctcggcgtttccaagtccgcg

SEQ ID NO: 28 - DNA, 34 bp, synthetic construct
  source 1..34: mol_type = other DNA
ctagaggatccccgggcaagaagactggaaaggt

SEQ ID NO: 29 - DNA, 34 bp, synthetic construct
  source 1..34: mol_type = other DNA
ctagaggatccccggaggcagttcgcgagagaat

SEQ ID NO: 30 - DNA, 34 bp, synthetic construct
  source 1..34: mol_type = other DNA
gctggtggaatatagatgtccgagcttaatgaaa

SEQ ID NO: 31 - DNA, 34 bp, synthetic construct
  source 1..34: mol_type = other DNA
gatccccgggtaccgttagaacattaccttatga

SEQ ID NO: 32 - DNA, 23 bp, synthetic construct
  source 1..23: mol_type = other DNA
cgcctataccaaaccagaagttg

SEQ ID NO: 33 - DNA, 18 bp, synthetic construct
  source 1..18: mol_type = other DNA
atggacgggataactttc

SEQ ID NO: 34 - DNA, 1095 bp, Candida boidinii B2
  source 1..1095: mol_type = genomic DNA
atgaaaatcgtgctggtgctgtacgacgcgggcaaacatgccgccgatgaagagaagctgtacggctgcaccgagaacaagctgggtatcgcgaactggctcaaagaccaaggccacgaactgatcacgacgagcgacaaagaaggcgagaccagcgaactggacaaacacatcccggacgcggatatcatcatcaccaccccgttccatccggcgtacatcaccaaagaacgtctggacaaggccaaaaatctgaagctggtggtggtggcgggcgttggcagtgaccacatcgacctcgactacattaaccagaccggcaaaaaaatcagcgtgctggaagtgaccggtagtaatgtggtgagcgtggccgagcacgtggtgatgaccatgctggtgctggtgcgcaactttgttccggcgcacgagcagatcatcaatcacgattgggaggtggccgccatcgcgaaggatgcctacgacatcgaaggcaaaaccatcgccaccattggtgcgggtcgcattggttaccgtgtgctggaacgtctgctgccattcaatccgaaggagctgctctactacgactaccaagccctcccgaaggaggcggaagaaaaagttggcgcgcgccgcgtggaaaacatcgaagaactggtggcccaagccgatatcgtgaccgtgaatgcgccactgcacgcgggtaccaaaggtctgatcaacaaggagctgctgagcaagttcaagaagggtgcgtggctggtgaatacggcccgtggtgcgatctgtgttgccgaggatgttgccgccgcgctggaaagtggtcaactgcgcggctacggtggcgatgtgtggttcccgcaaccggcgccaaaagatcatccgtggcgcgatatgcgcaataagtacggtgcgggcaatgcgatgaccccgcactatagcggtacgaccctcgatgcccaaacccgctacgcggaaggcacgaagaacatcctcgagagcttcttcaccggcaagtttgactaccgcccgcaagatatcattctgctgaacggtgaatacgtgaccaaggcctacggtaagcacgataagaaataa

SEQ ID NO: 35 - DNA, 2164 bp, synthetic construct
  source 1..2164: mol_type = other DNA
cgccgaccccatgtggtctcaagcccaaaggaagagtgaggcgagtcagtcgcgtaatgcttaggcacaggattgatttgtcgcaatgattgacacgattccgcttgacgctgcgtaaggtttttgtaattttacaggcaaccttttattcactaacaaatagctggtggaatatagatgaaaatcgtgctggtgctgtacgacgcgggcaaacatgccgccgatgaagagaagctgtacggctgcaccgagaacaagctgggtatcgcgaactggctcaaagaccaaggccacgaactgatcacgacgagcgacaaagaaggcgagaccagcgaactggacaaacacatcccggacgcggatatcatcatcaccaccccgttccatccggcgtacatcaccaaagaacgtctggacaaggccaaaaatctgaagctggtggtggtggcgggcgttggcagtgaccacatcgacctcgactacattaaccagaccggcaaaaaaatcagcgtgctggaagtgaccggtagtaatgtggtgagcgtggccgagcacgtggtgatgaccatgctggtgctggtgcgcaactttgttccggcgcacgagcagatcatcaatcacgattgggaggtggccgccatcgcgaaggatgcctacgacatcgaaggcaaaaccatcgccaccattggtgcgggtcgcattggttaccgtgtgctggaacgtctgctgccattcaatccgaaggagctgctctactacgactaccaagccctcccgaaggaggcggaagaaaaagttggcgcgcgccgcgtggaaaacatcgaagaactggtggcccaagccgatatcgtgaccgtgaatgcgccactgcacgcgggtaccaaaggtctgatcaacaaggagctgctgagcaagttcaagaagggtgcgtggctggtgaatacggcccgtggtgcgatctgtgttgccgaggatgttgccgccgcgctggaaagtggtcaactgcgcggctacggtggcgatgtgtggttcccgcaaccggcgccaaaagatcatccgtggcgcgatatgcgcaataagtacggtgcgggcaatgcgatgaccccgcactatagcggtacgaccctcgatgcccaaacccgctacgcggaaggcacgaagaacatcctcgagagcttcttcaccggcaagtttgactaccgcccgcaagatatcattctgctgaacggtgaatacgtgaccaaggcctacggtaagcacgataagaaataacggtaccctagctggtggaatatatgaaagtcgcagtcctcggcgctgctggcggtattggccaggcgcttgcactactgttaaaaacccaactgccttcaggttcagaactctctctgtatgatatcgctccagtgactcccggtgtggctgtcgatctgagccatatccctactgctgtgaaaatcaaaggtttttctggtgaagatgcgactccggcgctggaaggcgcagatgtcgttcttatctctgcaggcgtagcgcgtaaaccgggtatggatcgttccgacctgtttaacgttaacgccggcatcgtgaaaaacctggtacagcaagttgcgaaaacctgcccgaaagcgtgcattggtattatcactaacccggttaacaccacagttgcaattgctgctgaagtgctgaaaaaagccggtgtttatgacaaaaacaaactgttcggcgttaccacgctggatatcattcgttccaacacctttgttgcggaactgaaaggcaaacagccaggcgaagttgaagtgccggttattggcggtcactctggtgttaccattctgccgctgctgtcacaggttcctggcgttagttttaccgagcaggaagtggctgatctgaccaaacgcatccagaacgcgggtactgaagtggttgaagcgaaggccggtggcgggtctgcaaccctgtctatgggccaggcagctgcacgttttggtctgtctctggttcgtgcactgcagggcgaacaaggcgttgtcgaatgtgcctacgttgaaggcgacggtcagtacgcccgtttcttctctcaaccgctgctgctgggtaaaaacggcgtggaagagcgtaaatctatcggtaccctgagcgcatttgaacagaa

SEQ ID NO: 36 - DNA, 25 bp, synthetic construct
  source 1..25: mol_type = other DNA
cgccgaccccatgtggtctcaagcc

SEQ ID NO: 37 - DNA, 25 bp, synthetic construct
  source 1..25: mol_type = other DNA
ttctgttcaaatgcgctcagggtac

SEQ ID NO: 38 - DNA, 1650 bp, synthetic construct
  source 1..1650: mol_type = other DNA
aacgacggccagtgaattcgagctccgtaattgccctttaaaattcggggcgccgaccccatgtggtctcaagcccaaaggaagagtgaggcgagtcagtcgcgtaatgcttaggcacaggattgatttgtcgcaatgattgacacgattccgcttgacgctgcgtaaggtttttgtaattttacaggcaaccttttattcactaacaaatagctggtggaatatagatgaaaatcgtgctggtgctgtacgacgcgggcaaacatgccgccgatgaagagaagctgtacggctgcaccgagaacaagctgggtatcgcgaactggctcaaagaccaaggccacgaactgatcacgacgagcgacaaagaaggcgagaccagcgaactggacaaacacatcccggacgcggatatcatcatcaccaccccgttccatccggcgtacatcaccaaagaacgtctggacaaggccaaaaatctgaagctggtggtggtggcgggcgttggcagtgaccacatcgacctcgactacattaaccagaccggcaaaaaaatcagcgtgctggaagtgaccggtagtaatgtggtgagcgtggccgagcacgtggtgatgaccatgctggtgctggtgcgcaactttgttccggcgcacgagcagatcatcaatcacgattgggaggtggccgccatcgcgaaggatgcctacgacatcgaaggcaaaaccatcgccaccattggtgcgggtcgcattggttaccgtgtgctggaacgtctgctgccattcaatccgaaggagctgctctactacgactaccaagccctcccgaaggaggcggaagaaaaagttggcgcgcgccgcgtggaaaacatcgaagaactggtggcccaagccgatatcgtgaccgtgaatgcgccactgcacgcgggtaccaaaggtctgatcaacaaggagctgctgagcaagttcaagaagggtgcgtggctggtgaatacggcccgtggtgcgatctgtgttgccgaggatgttgccgccgcgctggaaagtggtcaactgcgcggctacggtggcgatgtgtggttcccgcaaccggcgccaaaagatcatccgtggcgcgatatgcgcaataagtacggtgcgggcaatgcgatgaccccgcactatagcggtacgaccctcgatgcccaaacccgctacgcggaaggcacgaagaacatcctcgagagcttcttcaccggcaagtttgactaccgcccgcaagatatcattctgctgaacggtgaatacgtgaccaaggcctacggtaagcacgataagaaataacggtaccctagctggtggaatatatgaaagtcgcagtcctcggcgctgctggcggtattggccaggcgcttgcactactgttaaaaacccaactgccttcaggttcagaactctctctgtatgatatcgctccagtgactcccggtgtggctgtcgatctgagccatatccctactgctgtgaaaatcaaaggtttttctggtgaagatgcgactccggcgctggaaggcgcagatgtcgttcttatctctgcaggcgtagcgcgtaaaccgggtatggatcgttccgacctgtttaacgttaacgccggcatcgtgaaaaacctggt

SEQ ID NO: 39 - DNA, 20 bp, synthetic construct
  source 1..20: mol_type = other DNA
aacgacggccagtgaattcg

SEQ ID NO: 40 - DNA, 21 bp, synthetic construct
  source 1..21: mol_type = other DNA
accaggtttttcacgatgccg

SEQ ID NO: 41 - protein, 312 aa, Escherichia coli str. K-12 substr. MG1655
MKVAVLGAAGGIGQALALLLKTQLPSGSELSLYDIAPVTPGVAVDLSHIPTAVKIKGFSGEDATPALEGADVVLISAGVARKPGMDRSDLFNVNAGIVKNLVQQVAKTCPKACIGIITNPVNTTVAIAAEVLKKAGVYDKNKLFGVTTLDIIRSNTFVAELKGKQPGEVEVPVIGGHSGVTILPLLSQVPGVSFTEQEVADLTKRIQNAGTEVVEAKAGGGSATLSMGQAAARFGLSLVRALQGEQGVVECAYVEGDGQYARFFSQPLLLGKNGVEERKSIGTLSAFEQNALEGMLDTLKKDIALGEEFVNK

SEQ ID NO: 42 - protein, 254 aa, Escherichia coli str. K-12 substr. MG1655 [sequence omitted]

SEQ ID NO: 43 - protein, 474 aa, Escherichia coli str. K-12 substr. MG1655 [sequence omitted]

SEQ ID NO: 44 - protein, 474 aa, Klebsiella pneumoniae subsp. pneumoniae MGH 78578
MSTEIKTQVVVLGAGPAGYSAAFRCADLGLETVIVERYSTLGGVCLNVGCIPSKALLHVAKVIEEAKALAEHGIVFGEPKTDIDKIRTWKEKVITQLTGGLAGMAKGRKVKVVNGLGKFTGANTLEVEGENGKTVINFDNAIIAAGSRPIQLPFIPHEDPRVWDSTDALELKSVPKRMLVMGGGIIGLEMGTVYHALGSEIDVVEMFDQVIPAADKDVVKVFTKRISKKFNLMLETKVTAVEAKEDGIYVSMEGKKAPAEAQRYDAVLVAIGRVPNGKNLDAGKAGVEVDDRGFIRVDKQMRTNVPHIFAIGDIVGQPMLAHKGVHEGHVAAEVISGLKHYFDPKVIPSIAYTEPEVAWVGLTEKEAKEKGISYETATFPWAASGRAIASDCADGMTKLIFDKETHRVIGGAIVGTNGGELLGEIGLAIEMGCDAEDIALTIHAHPTLHESVGLAAEVFEGSITDLPNAKAKKK

SEQ ID NO: 45 - protein, 760 aa, Escherichia coli str. K-12 substr. MG1655
MSELNEKLATAWEGFTKGDWQNEVNVRDFIQKNYTPYEGDESFLAGATEATTTLWDKVMEGVKLENRTHAPVDFDTAVASTITSHDAGYINKQLEKIVGLQTEAPLKRALIPFGGIKMIEGSCKAYNRELDPMIKKIFTEYRKTHNQGVFDVYTPDILRCRKSGVLTGLPDAYGRGRIIGDYRRVALYGIDYLMKDKLAQFTSLQADLENGVNLEQTIRLREEIAEQHRALGQMKEMAAKYGYDISGPATNAQEAIQWTYFGYLAAVKSQNGAAMSFGRTSTFLDVYIERDLKAGKITEQEAQEMVDHLVMKLRMVRFLRTPEYDELFSGDPIWATESIGGMGLDGRTLVTKNSFRFLNTLYTMGPSPEPNMTILWSEKLPLNFKKFAAKVSIDTSSLQYENDDLMRPDFNNDDYAIACCVSPMIVGKQMQFFGARANLAKTMLYAINGGVDEKLKMQVGPKSEPIKGDVLNYDEVMERMDHFMDWLAKQYITALNIIHYMHDKYSYEASLMALHDRDVIRTMACGIAGLSVAADSLSAIKYAKVKPIRDEDGLAIDFEIEGEYPQFGNNDPRVDDLAVDLVERFMKKIQKLHTYRDAIPTQSVLTITSNVVYGKKTGNTPDGRRAGAPFGPGANPMHGRDQKGAVASLTSVAKLPFAYAKDGISYTFSIVPNALGKDDEVRKTNLAGLMDGYFHHEASIEGGQHLNVNVMNREMLLDAMENPEKYPQLTIRVSGYAVRFNSLTKEQQQDVITRTFTQSM

SEQ ID NO: 46 - protein, 246 aa, Escherichia coli str. K-12 substr. MG1655
MSVIGRIHSFESCGTVDGPGIRFITFFQGCLMRCLYCHNRDTWDTHGGKEVTVEDLMKEVVTYRHFMNASGGGVTASGGEAILQAEFVRDWFRACKKEGIHTCLDTNGFVRRYDPVIDELLEVTDLVMLDLKQMNDEIHQNLVGVSNHRTLEFAKYLANKNVKVWIRYVVVPGWSDDDDSAHRLGEFTRDMGNVEKIELLPYHELGKHKWVAMGEEYKLDGVKPPKKETMERVKGILEQYGHKVMF

SEQ ID NO: 47 - protein, 364 aa, Candida boidinii B2
MKIVLVLYDAGKHAADEEKLYGCTENKLGIANWLKDQGHELITTSDKEGETSELDKHIPDADIIITTPFHPAYITKERLDKAKNLKLVVVAGVGSDHIDLDYINQTGKKISVLEVTGSNVVSVAEHVVMTMLVLVRNFVPAHEQIINHDWEVAAIAKDAYDIEGKTIATIGAGRIGYRVLERLLPFNPKELLYYDYQALPKEAEEKVGARRVENIEELVAQADIVTVNAPLHAGTKGLINKELLSKFKKGAWLVNTARGAICVAEDVAAALESGQLRGYGGDVWFPQPAPKDHPWRDMRNKYGAGNAMTPHYSGTTLDAQTRYAEGTKNILESFFTGKFDYRPQDIILLNGEYVTKAYGKHDKK